European Patent Application EP 4 560 005 A1, published May 28, 2025. Title: Novel strain of Schizochytrium sp. strain and a method for producing oil containing omega-3 using the same. Applicant: CJ CheilJedang Corporation. Application KR. The sequence listing filed with the application follows.

SEQUENCE LISTING (7 sequences)

SEQ ID NO: 1 - DNA, 850 bp, synthetic construct
  misc_feature 1..850: note = 18s rRNA sequence of CD01-1821
  source 1..850: mol_type = other DNA
aagcttgtttcaaagattaccatgcatgtgtaagtataagcgattgtactgtgagactgcgaacggctcattatatcagtaataatttcttcggtagtttcttttataggatacctgcagtaattctggaaataatacatgctgtaagagccctgtatggggctgcacttattagattgaagccgattttattggtgaatcatgataattgagcagattgacttttttgtcatgaatcgtttgagtttctgccccatcagttgtcacggtagtgtattggactacggtgactataacgggtgacggaagttagggctgactccggaagggagcctgaaacggctaccatatccaaggatagcacaggccgtaaattacccactgtggactccacaggtagtgacagaaatatcgatgcaagcgtgtatgcgttttgctatcggaatgaagcaatgtaaaaccctcatcgaggatcaactggagggcaagtctggtgccagcagccgcggtaattccagctccagaagcatatgctaaagttgttgcagttaaaaagctgtagttgaattttggcatgggcaccggtgctttccctgaatggggattgattgttgtgttgccttggccatctttttcttcttttttggaatctttcactgtaatcaaagcaagtgttccaagcaggcgatgaccggtatgtttattatgggatgataaataggacttgggtgctattttgttggtttgcacgcctgagtaaggttaataggaacagttgggggtattcgtatttaggagctagaggtgaaattcttgattccaaaagacaaacagaggaaaggcattccca

SEQ ID NO: 2 - DNA, 21 bp, synthetic construct
  misc_feature 1..21: note = Synthetic_18S-Fwd primer
  source 1..21: mol_type = other DNA
aacctggttgatcctgccagt

SEQ ID NO: 3 - DNA, 18 bp, synthetic construct
  misc_feature 1..18: note = Synthetic_LABY-ARev primer
  source 1..18: mol_type = other DNA
gggatcgaagatgattag

SEQ ID NO: 4 - DNA, 349 bp, synthetic construct
  misc_feature 1..349: note = DNA fragment sequence to be amplified of CD01-1821 strain
  source 1..349: mol_type = other DNA
gccaggcagctgaatgtaatgggatcacggcaagcttccaatacagattagaccgcccggatcccttacaaaaggctgtgaggccaatgatcgattgatcaatagatagttagatagatagatagatagatagatagatagatagatagatagatagatagatagatagatagatagatagatagatagatagatagatagatagatagatagatagatagatagatagatagaaaacaaatacctaggcgattactgcttcactatagcttttttctcctgcttttatccggctgccgtttcgaggcttgggcgaggcgccatttcccttcactcttctccacagcca

SEQ ID NO: 5 - DNA, 313 bp, synthetic construct
  misc_feature 1..313: note = DNA fragment sequence to be amplified of CD01-1003 strain
  source 1..313: mol_type = other DNA
gccaggcagctgaatgtaatgggatcacggcaagcttccaatacagattagaccgcccggatcccttacaaaaggctgtgaggccaatgatcgattgatcaatagatagttagatagatagatagatagatagatagatagatagatagatagatagatagatagatagatagatagatagatagatagatagatagaaaacaaatacctaggcgattactgcttcactatagcttttttctcctgcttttatccggctgccgtttcgaggcttgggcgaggcgccatttcccttcactcttctccacagcca

SEQ ID NO: 6 - DNA, 20 bp, synthetic construct
  misc_feature 1..20: note = synthetic_primer A
  source 1..20: mol_type = other DNA
gccaggcagctgaatgtaat

SEQ ID NO: 7 - DNA, 20 bp, synthetic construct
  misc_feature 1..20: note = synthetic_primer B
  source 1..20: mol_type = other DNA
tggctgtggagaagagtgaa